European Patent Application EP 4 467 549 A2, published November 27, 2024. Title: N-(3-(7H-pyrrolo[2,3-d]pyrimidin-4-yl)phenyl)benzamide Derivatives. Applicant: Novartis AG. The sequence listing filed with the application follows.

SEQUENCE LISTING (11 sequences)

SEQ ID NO: 1 - DNA, 44 bp, synthetic construct
  misc_feature 1..44: note = source = /note="Description of Artificial Sequence: Synthetic primer"
  source 1..44: mol_type = other DNA
cgatgaattcgccaccgctagcatggtgagcaagggcgaggagc

SEQ ID NO: 2 - DNA, 43 bp, synthetic construct
  misc_feature 1..43: note = source = /note="Description of Artificial Sequence: Synthetic primer"
  source 1..43: mol_type = other DNA
ctcattactaaccggctagcttacttgtacagctcgtccatgc

SEQ ID NO: 3 - DNA, 55 bp, synthetic construct
  misc_feature 1..55: note = source = /note="Description of Artificial Sequence: Synthetic primer"
  source 1..55: mol_type = other DNA
ccagcacagtggcggccgctcgagcatggtgagcaagggcgaggagctgttcacc

SEQ ID NO: 4 - DNA, 52 bp, synthetic construct
  misc_feature 1..52: note = source = /note="Description of Artificial Sequence: Synthetic primer"
  source 1..52: mol_type = other DNA
ccgcgggccctctagactcgagttacttgtacagctcgtccatgccgagagt

SEQ ID NO: 5 - DNA, 36 bp, synthetic construct
  misc_feature 1..36: note = source = /note="Description of Artificial Sequence: Synthetic primer"
  source 1..36: mol_type = other DNA
agagccctgctgaagttgaacccagctttcttgtac

SEQ ID NO: 6 - DNA, 36 bp, synthetic construct
  misc_feature 1..36: note = source = /note="Description of Artificial Sequence: Synthetic primer"
  source 1..36: mol_type = other DNA
gtacaagaaagctgggttcaacttcagcagggctct

SEQ ID NO: 7 - DNA, 39 bp, synthetic construct
  misc_feature 1..39: note = source = /note="Description of Artificial Sequence: Synthetic primer"
  source 1..39: mol_type = other DNA
gagtacatggccaatggctccctcctgaactacctgagg

SEQ ID NO: 8 - DNA, 39 bp, synthetic construct
  misc_feature 1..39: note = source = /note="Description of Artificial Sequence: Synthetic primer"
  source 1..39: mol_type = other DNA
cctcaggtagttcaggagggagccattggccatgtactc

SEQ ID NO: 9 - DNA, 1551 bp, synthetic construct
  misc_feature 1..1551: note = source = /note="Description of Artificial Sequence: Synthetic polynucleotide"
  source 1..1551: mol_type = other DNA
gatatccagcacagtggcggccgctcgagcatggtgagcaagggcgaggagctgttcaccggggtggtgcccatcctggtcgagctggacggcgacgtaaacggccacaagttcagcgtgtccggcgagggcgagggcgatgccacctacggcaagctgaccctgaagttcatctgcaccaccggcaagctgcccgtgccctggcccaccctcgtgaccaccctgacctacggcgtgcagtgcttcagccgctaccccgaccacatgaagcagcacgacttcttcaagtccgccatgcccgaaggctacgtccaggagcgcaccatcttcttcaaggacgacggcaactacaagacccgcgccgaggtgaagttcgagggcgacaccctggtgaaccgcatcgagctgaagggcatcgacttcaaggaggacggcaacatcctggggcacaagctggagtacaactacaacagccacaacgtctatatcatggccgacaagcagaagaacggcatcaaggtgaacttcaagatccgccacaacatcgaggacggcagcgtgcagctcgccgaccactaccagcagaacacccccatcggcgacggccccgtgctgctgcccgacaaccactacctgagcacccagtccgccctgagcaaagaccccaacgagaagcgcgatcacatggtcctgctggagttcgtgaccgccgccgggatcactctcggcatggacgagctgtacaagggaagcggagcgacgaattttagtctactgaaacaagcgggagacgtggaggaaaaccctggacctatggtgagcaagggcgaggaggataacatggccatcatcaaggagttcatgcgcttcaaggtgcacatggagggctccgtgaacggccacgagttcgagatcgagggcgagggcgagggccgcccctacgagggcacccagaccgccaagctgaaggtgaccaagggtggccccctgcccttcgcctgggacatcctgtcccctcagttcatgtacggctccaaggcctacgtgaagcaccccgccgacatccccgactacttgaagctgtccttccccgagggcttcaagtgggagcgcgtgatgaacttcgaggacggcggcgtggtgaccgtgacccaggactcctccctgcaggacggcgagttcatctacaaggtgaagctgcgcggcaccaacttcccctccgacggccccgtaatgcagaagaagaccatgggctgggaggcctcctccgagcggatgtaccccgaggacggcgccctgaagggcgagatcaagcagaggctgaagctgaaggacggcggccactacgacgctgaggtcaagaccacctacaaggccaagaagcccgtgcagctgcccggcgcctacaacgtcaacatcaagttggacatcacctcccacaacgaggactacaccatcgtggaacagtacgaacgcgccgagggccgccactccaccggcggcatggacgagctgtacaagtagctcgagtctagagggcccgcggttaac

SEQ ID NO: 10 - DNA, 39 bp, synthetic construct
  misc_feature 1..39: note = source = /note="Description of Artificial Sequence: Synthetic primer"
  source 1..39: mol_type = other DNA
gtcatggatgaagaatccttgaacccagctttcttgtac

SEQ ID NO: 11 - DNA, 39 bp, synthetic construct
  misc_feature 1..39: note = source = /note="Description of Artificial Sequence: Synthetic primer"
  source 1..39: mol_type = other DNA
gtacaagaaagctgggttcaaggattcttcatccatgac